European Patent Application EP 4 327 826 A1, published February 28, 2024. Title: Pharmaceuticals for use in combination for prophylaxis and/or treatment of dyslipidemia or cardiovascular events. Applicant: KOWA COMPANY, LTD. The sequence listing filed with the application follows.

SEQUENCE LISTING (4 sequences)

SEQ ID NO: 1 - DNA, 20 bp, Artificial Sequence
  Forward primer for Ppara gene
tcatactcgcaggaaagact

SEQ ID NO: 2 - DNA, 20 bp, Artificial Sequence
  Reverse primer for Ppara gene
acctctgcctccttgttttc

SEQ ID NO: 3 - DNA, 20 bp, Artificial Sequence
  Forward primer for Beta-actin gene
agccatgtacgtagccatcc

SEQ ID NO: 4 - DNA, 20 bp, Artificial Sequence
  Reverse primer for Beta-actin gene
accctcatagatgggcacag